European Patent Application EP 4 174 183 A1, published May 3, 2023. Title: FUSION GENE, RECOMBINANT NOVEL CORONAVIRUS HIGH-EFFICIENCY IMMUNE DNA VACCINE, CONSTRUCTION METHOD AND USE THEREOF. Applicant: Aurora Genevac Biotech Co., Ltd. The sequence listing filed with the application follows.

SEQUENCE LISTING (15 sequences)

SEQ ID NO: 1 - DNA, 14441 bp, Artificial Sequence
gcttactggcttatcgaaattaatacgactcactatagggagaccggaagcttgaattcatggcggatgtgtgacatacacgacgccaaaagattttgttccagctcctgccacctccgctacgcgagagattaaccacccacgatggccgccaaagtgcatgttgatattgaggctgacagcccattcatcaagtctttgcagaaggcatttccgtcgttcgaggtggagtcattgcaggtcacaccaaatgaccatgcaaatgccagagcattttcgcacctggctaccaaattgatcgagcaggagactgacaaagacacactcatcttggatatcggcagtgcgccttccaggagaatgatgtctacgcacaaataccactgcgtatgccctatgcgcagcgcagaagaccccgaaaggctcgtatgctacgcaaagaaactggcagcggcctccgggaaggtgctggatagagagatcgcaggaaaaatcaccgacctgcagaccgtcatggctacgccagacgctgaatctcctaccttttgcctgcatacagacgtcacgtgtcgtacggcagccgaagtggccgtataccaggacgtgtatgctgtacatgcaccaacatcgctgtaccatcaggcgatgaaaggtgtcagaacggcgtattggattgggtttgacaccaccccgtttatgtttgacgcgctagcaggcgcgtatccaacctacgccacaaactgggccgacgagcaggtgttacaggccaggaacataggactgtgtgcagcatccttgactgagggaagactcggcaaactgtccattctccgcaagaagcaattgaaaccttgcgacacagtcatgttctcggtaggatctacattgtacactgagagcagaaagctactgaggagctggcacttaccctccgtattccacctgaaaggtaaacaatcctttacctgtaggtgcgataccatcgtatcatgtgaagggtacgtagttaagaaaatcactatgtgccccggcctgtacggtaaaacggtagggtacgccgtgacgtatcacgcggagggattcctagtgtgcaagaccacagacactgtcaaaggagaaagagtctcattccctgtatgcacctacgtcccctcaaccatctgtgatcaaatgactggcatactagcgaccgacgtcacaccggaggacgcacagaagttgttagtgggattgaatcagaggatagttgtgaacggaagaacacagcgaaacactaacacgatgaagaactatctgcttccgattgtggccgtcgcatttagcaagtgggcgagggaatacaaggcagaccttgatgatgaaaaacctctgggtgtccgagagaggtcacttacttgctgctgcttgtgggcatttaaaacgaggaagatgcacaccatgtacaagaaaccagacacccagacaatagtgaaggtgccttcagagtttaactcgttcgtcatcccgagcctatggtctacaggcctcgcaatcccagtcagatcacgcattaagatgcttttggccaagaagaccaagcgagagttaatacctgttctcgacgcgtcgtcagccagggatgctgaacaagaggagaaggagaggttggaggccgagctgactagagaagccttaccacccctcgtccccatcgcgccggcggagacgggagtcgtcgacgtcgacgttgaagaactagagtatcacgcaggtgcaggggtcgtggaaacacctcgcagcgcgttgaaagtcaccgcacagccgaacgacgtactactaggaaattacgtagttctgtccccgcagaccgtgctcaagagctccaagttggcccccgtgcaccctctagcagagcaggtgaaaataataacacataacgggagggccggccgttaccaggtcgacggatatgacggcagggtcctactaccatgtggatcggccattccggtccctgagtttcaagctttgagcgagagcgccactatggtgtacaacgaaagggagttcgtcaacaggaaactataccatattgccgttcacggaccgtcgctgaacaccgacgaggagaactacgagaaagtcagagctgaaagaactgacgccgagtacgtgttcgacgtagataaaaaatgctgcgtcaagagagaggaagcgtcgggtttggtgttggtgggagagctaaccaaccccccgttccatgaattcgcctacgaagggctgaagatcaggccgtcggcaccatataagactacagtagtaggagtctttggggttccgggatcaggcaagtctgctattattaagagcctcgtgaccaaacacgatctggtcaccagcggcaagaaggagaactgccaggaaatagtcaacgacgtgaagaagcaccgcggactggacatccaggcaaaaacagtggactccatcctgctaaacgggtgtcgtcgtgccgtggacatcctatatgtggacgaggctttcgcttgccattccggtactctgctagccctaattgctcttgttaaacctcggagcaaagtggtgttatgcggagaccccaagcaatgcggattcttcaatatgatgcagcttaaggtgaacttcaaccacaacatctgcactgaagtatgtcataaaagtatatccagacgttgcacgcgtccagtcacggccatcgtgtctacgttgcactacggaggcaagatgcgcacgaccaacccgtgcaacaaacccataatcatagacaccacaggacagaccaagcccaagccaggagacatcgtgttaacatgcttccgaggctgggtaaagcagctgcagttggactaccgtggacacgaagtcatgacagcagcagcatctcagggcctcacccgcaaaggggtatacgccgtaaggcagaaggtgaatgaaaatcccttgtatgcccctgcgtcggagcacgtgaatgtactgctgacgcgcactgaggataggctggtgtggaaaacgctggccggcgatccctggattaaggtcctatcaaacattccacagggtaactttacggccacattggaagaatggcaagaagaacacgacaaaataatgaaggtgattgaaggaccggctgcgcctgtggacgcgttccagaacaaagcgaacgtgtgttgggcgaaaagcctggtgcctgtcctggacactgccggaatcagattgacagcagaggagtggagcaccataattacagcatttaaggaggacagagcttactctccagtggtggccttgaatgaaatttgcaccaagtactatggagttgacctggacagtggcctgttttctgccccgaaggtgtccctgtattacgagaacaaccactgggataacagacctggtggaaggatgtatggattcaatgccgcaacagctgccaggctggaagctagacataccttcctgaaggggcagtggcatacgggcaagcaggcagttatcgcagaaagaaaaatccaaccgctttctgtgctggacaatgtaattcctatcaaccgcaggctgccgcacgccctggtggctgagtacaagacggttaaaggcagtagggttgagtggctggtcaataaagtaagagggtaccacgtcctgctggtgagtgagtacaacctggctttgcctcgacgcagggtcacttggttgtcaccgctgaatgtcacaggcgccgataggtgctacgacctaagtttaggactgccggctgacgccggcaggttcgacttggtctttgtgaacattcacacggaattcagaatccaccactaccagcagtgtgtcgaccacgccatgaagctgcagatgcttgggggagatgcgctacgactgctaaaacccggcggcagcctcttgatgagagcttacggatacgccgataaaatcagcgaagccgttgtttcctccttaagcagaaagttctcgtctgcaagagtgttgcgcccggattgtgtcaccagcaatacagaagtgttcttgctgttctccaactttgacaacggaaagagaccctctacgctacaccagatgaataccaagctgagtgccgtgtatgccggagaagccatgcacacggccgggtgtgcaccatcctacagagttaagagagcagacatagccacgtgcacagaagcggctgtggttaacgcagctaacgcccgtggaactgtaggggatggcgtatgcagggccgtggcgaagaaatggccgtcagcctttaagggagaagcaacaccagtgggcacaattaaaacagtcatgtgcggctcgtaccccgtcatccacgctgtagcgcctaatttctctgccacgactgaagcggaaggggaccgcgaattggccgctgtctaccgggcagtggccgccgaagtaaacagactgtcactgagcagcgtagccatcccgctgctgtccacaggagtgttcagcggcggaagagataggctgcagcaatccctcaaccatctattcacagcaatggacgccacggacgctgacgtgaccatctactgcagagacaaaagttgggagaagaaaatccaggaagccatagacatgaggacggctgtggagttgctcaatgatgacgtggagctgaccacagacttggtgagagtgcacccggacagcagcctggtgggtcgtaagggctacagtaccactgacgggtcgctgtactcgtactttgaaggtacgaaattcaaccaggctgctattgatatggcagagatactgacgttgtggcccagactgcaagaggcaaacgaacagatatgcctatacgcgctgggcgaaacaatggacaacatcagatccaaatgtccggtgaacgattccgattcatcaacacctcccaggacagtgccctgcctgtgccgctacgcaatgacagcagaacggatcgcccgccttaggtcacaccaagttaaaagcatggtggtttgctcatcttttcccctcccgaaataccatgtagatggggtgcagaaggtaaagtgcgagaaggttctcctgttcgacccgacggtaccttcagtggttagtccgcggaagtatgccgcatctacgacggaccactcagatcggtcgttacgagggtttgacttggactggaccaccgactcgtcttccactgccagcgataccatgtcgctacccagtttgcagtcgtgtgacatcgactcgatctacgagccaatggctcccatagtagtgacggctgacgtacaccctgaacccgcaggcatcgcggacctggcggcagatgtgcatcctgaacccgcagaccatgtggacctcgagaacccgattcctccaccgcgcccgaagagagctgcataccttgcctcccgcgcggcggagcgaccggtgccggcgccgagaaagccgacgcctgccccaaggactgcgtttaggaacaagctgcctttgacgttcggcgactttgacgagcacgaggtcgatgcgttggcctccgggattactttcggagacttcgacgacgtcctgcgactaggccgcgcgggtgcatatattttctcctcggacactggcagcggacatttacaacaaaaatccgttaggcagcacaatctccagtgcgcacaactggatgcggtcgaggaggagaaaatgtacccgccaaaattggatactgagagggagaagctgttgctgctgaaaatgcagatgcacccatcggaggctaataagagtcgataccagtctcgcaaagtggagaacatgaaagccacggtggtggacaggctcacatcgggggccagattgtacacgggagcggacgtaggccgcataccaacatacgcggttcggtacccccgccccgtgtactcccctaccgtgatcgaaagattctcaagccccgatgtagcaatcgcagcgtgcaacgaatacctatccagaaattacccaacagtggcgtcgtaccagataacagatgaatacgacgcatacttggacatggttgacgggtcggatagttgcttggacagagcgacattctgcccggcgaagctccggtgctacccgaaacatcatgcgtaccaccagccgactgtacgcagtgccgtcccgtcaccctttcagaacacactacagaacgtgctagcggccgccaccaagagaaactgcaacgtcacgcaaatgcgagaactacccaccatggactcggcagtgttcaacgtggagtgcttcaagcgctatgcctgctccggagaatattgggaagaatatgctaaacaacctatccggataaccactgagaacatcactacctatgtgaccaaattgaaaggcccgaaagctgctgccttgttcgctaagacccacaacttggttccgctgcaggaggttcccatggacagattcacggtcgacatgaaacgagatgtcaaagtcactccagggacgaaacacacagaggaaagacccaaagtccaggtaattcaagcagcggagccattggcgaccgcttacctgtgcggcatccacagggaattagtaaggagactaaatgctgtgttacgccctaacgtgcacacattgtttgatatgtcggccgaagactttgacgcgatcatcgcctctcacttccacccaggagacccggttctagagacggacattgcatcattcgacaaaagccaggacgactccttggctcttacaggtttaatgatcctcgaagatctaggggtggatcagtacctgctggacttgatcgaggcagcctttggggaaatatccagctgtcacctaccaactggcacgcgcttcaagttcggagctatgatgaaatcgggcatgtttctgactttgtttattaacactgttttgaacatcaccatagcaagcagggtactggagcagagactcactgactccgcctgtgcggccttcatcggcgacgacaacatcgttcacggagtgatctccgacaagctgatggcggagaggtgcgcgtcgtgggtcaacatggaggtgaagatcattgacgctgtcatgggcgaaaaacccccatatttttgtgggggattcatagtttttgacagcgtcacacagaccgcctgccgtgtttcagacccacttaagcgcctgttcaagttgggtaagccgctaacagctgaagacaagcaggacgaagacaggcgacgagcactgagtgacgaggttagcaagtggttccggacaggcttgggggccgaactggaggtggcactaacatctaggtatgaggtagagggctgcaaaagtatcctcatagccatggccaccttggcgagggacattaaggcgtttaagaaattgagaggacctgttatacacctctacggcggtcctagattggtgcgttaatacacagaattctgattggatcccgccaccatgatcaagctgaagttcggggtgttcttcaccgtgctgctgagcagcgcctacgcccacgggacccctcagaacatcaccgacctgtgcgccgagtaccacaacacccagatctacaccctgaacgacaagattttcagctacaccgaaagcctggcaggaaaaagagagatggccatcatcaccttcaaaaacggcgccatcttccaggtggaggtgcccggcagccagcacatcgatagccagaagaaggccatcgaaagaatgaaggacacactgagaatcgcctacctgaccgaggccaaggtggaaaagctgtgcgtgtggaataataagaccccccacgccatcgccgccatcagcatggccaaccagtacatcaaggcaaacagcaaattcatcggaatcaccgaaaaagccatgcacgtggcacagcccgccgtggtgctggcaagctccagaggaatcgcctccttcgtgtgcgagtacgccagccccggaaaggccacagaggtgagagtgaccgtgctgagacaggccgactcccaggtgaccgaagtgtgtgctgccacatacatgatgggcaacgagctgaccttcctggacgattccatctgcaccggaaccagcagtggaaaccaggtgaacctgaccattcagggcctgagggccatggacaccggactgtacatctgcaaggtggagctgatgtacccccccccctactacctgggcatcggaaacggaacccagatctatgtgatcgaccccgagccatgtcccgacagcgactttaccgtgaccgtgcccaaggacctgtacgtggtggagtacggctctaacatgaccatcgagtgtaaatttcccgtggagaagcagctggacctggcagccctgatcgtgtactgggagatggaggacaagaacatcatccagtttgtgcacggcgaggaagacctgaaggtgcagcactcctcatacagacagagagccagactgctgaaagaccagctgagcctgggcaacgcagccctgcagatcaccgacgtgaagctgcaggacgccggagtgtacagatgcatgatcagctacggaggggcagactacaagagaatcaccgtgaaagtgaacgcaccctacaacaaaatcaaccagagaatcctggtggtggaccccgtgaccagcgagcacgagctgacctgccaggccgagggctaccccaaggcagaggtgatctggaccagcagcgaccaccaggtgctgagcggcaagaccaccaccaccaatagcaaaagagaggaaaagctgttcaacgtgaccagcacactgagaattaatacaaccaccaacgagatcttctactgcacattcagaagactggaccccgaagaaaaccacaccgccgagctggtgatccccgaactgcccctggcccacccccctaacgaaagaacccacctggtgatcctgggcgccatcctgctgtgcctgggagtggccctgaccttcatcttccgcctgagaaagggcaggatgatggacgtgaaaaagtgcggcatccaggacacaaacagcaaaaagcagagcgatacccacctggaggagaccgccaaatttgtggccgcctggaccctgaaggcagccgcttgagaattcggcccctctccctcccccccccctaacgttactggccgaagccgcttggaataaggccggtgtgcgtttgtctatatgttattttccaccatattgccgtcttttggcaatgtgagggcccggaaacctggccctgtcttcttgacgagcattcctaggggtctttcccctctcgccaaaggaatgcaaggtctgttgaatgtcgtgaaggaagcagttcctctggaagcttcttgaagacaaacaacgtctgtagcgaccctttgcaggcagcggaaccccccacctggcgacaggtgcctctgcggccaaaagccacgtgtataagatacacctgcaaaggcggcacaaccccagtgccacgttgtgagttggatagttgtggaaagagtcaaatggctctcctcaagcgtattcaacaaggggctgaaggatgcccagaaggtaccccattgtatgggatctgatctggggcctcggtgcacatgctttacatgtgtttagtcgaggttaaaaaaacgtctaggccccccgaaccacggggacgtggttttcctttgaaaaacacgatgataagcttgccacaacccgcgcgcttaattaacccggggccaccatggagcgggtgcagcccctggaggagaacgtgggcaacgccgccagacccaggttcgagagaaacaagctgctgctggtggccagcgtgatccagggactgggcctgctgctgtgcttcacctatatttgcctgcactttagtgccctgcaggtgagtcatagatacccccgcattcagtccatcaaagtgcagttcaccgagtataagaaggagaagggattcattctgacctcccagaaggaggacgagatcatgaaggtgcagaacaatagcgtgatcatcaactgtgacggcttttacctgatttcactgaaaggatacttcagccaggaggtgaatatcagcctgcactaccagaaagacgaggagcccctgttccagctgaagaaggtgaggagcgtgaacagcctgatggtggccagcctgacctacaaggacaaagtgtacctgaacgtgaccaccgacaacaccagcctggatgattttcacgtgaacggaggcgagctgatcctgatccatcagaaccccggcgagttctaagggtaattaattgacgttttacggccgccggtggcgcccgcgcccggcggcccgtccctggccgttgcaggccactccggtggctcccgtcgtccccgacttccaggcccagcagatgcagcaactcatcagcgccgtaaatgcgctgacaatgagacagaacgcaattgctcctgctaggcctcccaaaccaaagaagaagaagacaaccaaaccaaagccgaaaacgcagcccaagaagatcaacggaaaaacgcagcagcaaaagaagaaagacaagcaagccgacaagaagaagaagaaacccggaaaaagagaaagaatgtgcatgaagattgaaaatgactgtatcttcgtatgcggctagccacagtaacgtagtgtttccagacatgtcgggcaccgcactatcatgggtgcagaaaatctcgggtggtctgggggccttcgcaatcggcgctatcctggtgctggttgtggtcacttgcattgggctccgcagataagttagggtaggcaatggcattgatatagcaagaaaattgaaaacagaaaaagttagggtaagcaatggcatataaccataactgtataacttgtaacaaagcgcaacaagacctgcgcaattggccccgtggtccgcctcacggaaactcggggcaactcatattgacacattaattggcaataattggaagcttacataagcttaattcgacgaataattggatttttattttattttgcaattggtttttaatatttccaaaaaaaaaaaaaaaaaaaaaaaaaaaaaaaaaaaaaaaaaaaaaaaaaaaaaaaaaactagagatcataatcagccatatcacatctgtagaggttttacttgctttaaaaaacctcccacacctccccctgaacctgaaacataaaatgaatgcaattgttgttgttaacttgtttattgcagcttataatggttacaaataaagcaatagcatcacaaatttcacaaataaagcatttttttcactgcattctagttgtggtttgtccaaactcatcaatgtatcttatcatgtctggatctagtctgcattaatgaatcggccaacgcgcggggagaggcggtttgcgtattgggcgctcttccgcttcctcgctcactgactcgctgcgctcggtcgttcggctgcggcgagcggtatcagctcactcaaaggcggtaatacggttatccacagaatcaggggataacgcaggaaagaacatgtgagcaaaaggccagcaaaaggccaggaaccgtaaaaaggccgcgttgctggcgtttttccataggctccgcccccctgacgagcatcacaaaaatcgacgctcaagtcagaggtggcgaaacccgacaggactataaagataccaggcgtttccccctggaagctccctcgtgcgctctcctgttccgaccctgccgcttaccggatacctgtccgcctttctcccttcgggaagcgtggcgctttctcatagctcacgctgtaggtatctcagttcggtgtaggtcgttcgctccaagctgggctgtgtgcacgaaccccccgttcagcccgaccgctgcgccttatccggtaactatcgtcttgagtccaacccggtaagacacgacttatcgccactggcagcagccactggtaacaggattagcagagcgaggtatgtaggcggtgctacagagttcttgaagtggtggcctaactacggctacactagaagaacagtatttggtatctgcgctctgctgaagccagttaccttcggaaaaagagttggtagctcttgatccggcaaacaaaccaccgctggtagcggtggtttttttgtttgcaagcagcagattacgcgcagaaaaaaaggatctcaagaagatcctttgatcttttctacggggtctgacgctcagtggaacgaaaactcacgttaagggattttggtcatgagattatcaaaaaggatcttcacctagatccttttaaattaaaaatgaagttttaaatcaatctaaagtatatatgagtaaacttggtctgacagactagtatgattgaacaagatggattgcacgcaggttctccggccgcttgggtggagaggctattcggctatgactgggcacaacagacaatcggctgctctgatgccgccgtgttccggctgtcagcgcaggggcgcccggttctttttgtcaagaccgacctgtccggtgccctgaatgaactgcaagacgaggcagcgcggctatcgtggctggccacgacgggcgttccttgcgcagctgtgctcgacgttgtcactgaagcgggaagggactggctgctattgggcgaagtgccggggcaggatctcctgtcatctcaccttgctcctgccgagaaagtatccatcatggctgatgcaatgcggcggctgcatacgcttgatccggctacctgcccattcgaccaccaagcgaaacatcgcatcgagcgagcacgtactcggatggaagccggtcttgtcgatcaggatgatctggacgaagagcatcaggggctcgcgccagccgaactgttcgccaggctcaaggcgagtatgcccgacggcgaggatctcgtcgtgacccatggcgatgcctgcttgccgaatatcatggtggaaaatggccgcttttctggattcatcgactgtggccggctgggtgtggcggaccgctatcaggacatagcgttggctacccgtgatattgctgaagagcttggcggcgaatgggctgaccgcttcctcgtgctttacggtatcgccgctcccgattcgcagcgcatcgccttctatcgccttcttgacgagttcttctgactcgaggcatgcaccatgattacgaattcacgcgtgcatgctcgggggacgatcgtcggggggctcgggggacgatcgtcggggggctcgggggacgatcgtcggggggctcgggggacgatcgtcggggggctcgggcatgcacgcgtaagcttggcactggccgaccatgattacgaattcacgcgtgcatgctcgggggacgatcgtcggggggctcgggggacgatcgtcggggggctcgggggacgatcgtcggggggctcgggggacgatcgtcggggggctcgggcatgcacgcgtaagcttggcactggccggcatgcaagctgcaggcatgcaccatgattacgaattcacgcgtgcatgctcgggggacgatcgtcggggggctcgggggacgatcgtcggggggctcgggggacgatcgtcggggggctcgggggacgatcgtcggggggctcgggcatgcacgcgtaagcttggcactggccgaccatgattacgaattcacgcgtgcatgctcgggggacgatcgtcggggggctcgggggacgatcgtcggggggctcgggggacgatcgtcggggggctcgggggacgatcgtcggggggctcgggcatgcacgcgtaagcttggcactggccggcatgcaagctcggatccaccggtcgccaccatggtgagcaacatgcaagctcgtaatcaattacggggtcattagttcatagcccatatatggagttccgcgttacataacttacggtaaatggcccgcctggctgaccgcccaacgacccccgcccattgacgtcaataatgacgtatgttcccatagtaacgccaatagggactttccattgacgtcaatgggtggagtatttacggtaaactgcccacttggcagtacatcaagtgtatcatatgccaagtacgccccctattgacgtcaatgacggtaaatggcccgcctggcattatgcccagtacatgaccttatgggactttcctacttggcagtacatctacgtattagtcatcgctattaccatggtgatgcggttttggcagtacatcaatgggcgtggatagcggtttgactcacggggatttccaagtctccaccccattgacgtcaatgggagtttgttttggcaccaaaatcaacgggactttccaaaatgtcgtaacaactccgccccattgacgcaaatgggcggtaggcgtgtacggtgggaggtctatataagcagagctctctggctaactagagaacccact

SEQ ID NO: 2 - DNA, 372 bp, Artificial Sequence
atgatcaagctgaagttcggggtgttcttcaccgtgctgctgagcagcgcctacgcccacgggacccctcagaacatcaccgacctgtgcgccgagtaccacaacacccagatctacaccctgaacgacaagattttcagctacaccgaaagcctggcaggaaaaagagagatggccatcatcaccttcaaaaacggcgccatcttccaggtggaggtgcccggcagccagcacatcgatagccagaagaaggccatcgaaagaatgaaggacacactgagaatcgcctacctgaccgaggccaaggtggaaaagctgtgcgtgtggaataataagaccccccacgccatcgccgccatcagcatggccaac

SEQ ID NO: 3 - DNA, 42 bp, Artificial Sequence
cagtacatcaaggcaaacagcaaattcatcggaatcaccgaa

SEQ ID NO: 4 - DNA, 39 bp, Artificial Sequence
gccaaatttgtggccgcctggaccctgaaggcagccgct

SEQ ID NO: 5 - DNA, 18 bp, Artificial Sequence
ggcggcggcggcggcggc

SEQ ID NO: 6 - DNA, 1413 bp, Artificial Sequence
cgcgtgcagcccaccgagagcatcgtgcgcttccccaacatcaccaacctgtgccccttcggcgaggtgttcaacgccacccgcttcgccagcgtgtacgcctggaaccgcaagcgcatcagcaactgcgtggccgactacagcgtgctgtacaacagcgccagcttcagcaccttcaagtgctacggcgtgagccccaccaagctgaacgacctgtgcttcaccaacgtgtacgccgacagcttcgtgatccgcggcgacgaggtgcgccagatcgcccccggccagaccggcaagatcgccgactacaactacaagctgcccgacgacttcaccggctgcgtgatcgcctggaacagcaacaacctggacagcaaggtgggcggcaactacaactacctgtaccgcctgttccgcaagagcaacctgaagcccttcgagcgcgacatcagcaccgagatctaccaggccggcagcaccccctgcaacggcgtggagggcttcaactgctacttccccctgcagagctacggcttccagcccaccaacggcgtgggctaccagccctaccgcgtggtggtgctgagcttcgagctgctgcacgcccccgccaccgtgtgcggccccaagaagagcaccaacctggtgaagaacaagtgcgtgaacttcggcggcggcggcagcggcggcggcggcagcgtgctgaacgacatcctgagccgcctggacaaggtggaggccgaggtgcagatcgaccgcctgatcaccggccgcctgcagagcctgcagacctacgtgacccagcagctgatccgcgccgccgagatccgcgccagcgccaacctggccgccaccaagatgagcgagtgcgtgctgggccagagcaagcgcgtggacttctgcggcaagggctaccacctgatgagcttcccccagagcgccccccacggcgtggtgttcctgcacgtgacctacgtgcccgcccaggagaagaacttcaccaccgcccccgccatctgccacgacggcaaggcccacttcccccgcgagggcgtgttcgtgagcaacggcacccactggttcgtgacccagcgcaacttctacgagccccagatcatcaccaccgacaacaccttcgtgagcggcaactgcgacgtggtgatcggcatcgtgaacaacaccgtgtacgaccccctgcagcccgagctggacagcttcaaggaggagctggacaagtacttcaagaaccacaccagccccgacgtggacctgggcgacatcagcggcatcaacgccagcgtggtgaacatccagaaggagatcgaccgcctgaacgaggtggccaagaacctgaacgagagcctgatcgacctgcaggagctgggcaagtacgagcagtacatcaagtggccc

SEQ ID NO: 7 - DNA, 96 bp, Artificial Sequence
ggctacatccccgaggccccccgcgacggccaggcctacgtgcgcaaggacggcgagtgggtgctgctgagcaccttcctgtgccccccctgcccc

SEQ ID NO: 8 - DNA, 84 bp, Artificial Sequence
cgcgccaagcgcgcccccgtgaagcagaccctgaacttcgacctgctgaagctggccggcgacgtggagagcaaccccggcccc

SEQ ID NO: 9 - DNA, 51 bp, Artificial Sequence
atgcgctacatgatcctgggcctgctggccctggccgccgtgtgcagcgcc

SEQ ID NO: 10 - DNA, 699 bp, Artificial Sequence
gccctgaacacccccaaggaccacatcggcacccgcaaccccgccaacaacgccgccatcgtgctgcagctgccccagggcaccaccctgcccaagggcttctacgccgagggcagccgcggcggcagccaggccagcagccgcagcagcagccgcagccgcaacagcagccgcaacagcacccccggcagcagccgcggcaccagccccgcccgcatggccggcaacggcggcgacgccgccctggccctgctgctgctggaccgcctgaaccagctggagagcaagatgagcggcaagggccagcagcagcagggccagaccgtgaccaagaagagcgccgccgaggccagcaagaagccccgccagaagcgcaccgccaccaaggcctacaacgtgacccaggccttcggccgccgcggccccgagcagacccagggcaacttcggcgaccaggagctgatccgccagggcaccgactacaagcactggccccagatcgcccagttcgcccccagcgccagcgccttcttcggcatgagccgcatcggcatggaggtgacccccagcggcacctggctgacctacaccggcgccatcaagctggacgacaaggaccccaacttcaaggaccaggtgatcctgctgaacaagcacatcgacgcctacaagaccttcccccccaccgagcccaagtga

SEQ ID NO: 11 - DNA, 569 bp, Artificial Sequence
gcccctctccctcccccccccctaacgttactggccgaagccgcttggaataaggccggtgtgcgtttgtctatatgttattttccaccatattgccgtcttttggcaatgtgagggcccggaaacctggccctgtcttcttgacgagcattcctaggggtctttcccctctcgccaaaggaatgcaaggtctgttgaatgtcgtgaaggaagcagttcctctggaagcttcttgaagacaaacaacgtctgtagcgaccctttgcaggcagcggaaccccccacctggcgacaggtgcctctgcggccaaaagccacgtgtataagatacacctgcaaaggcggcacaaccccagtgccacgttgtgagttggatagttgtggaaagagtcaaatggctctcctcaagcgtattcaacaaggggctgaaggatgcccagaaggtaccccattgtatgggatctgatctggggcctcggtgcacatgctttacatgtgtttagtcgaggttaaaaaaacgtctaggccccccgaaccacggggacgtggttttcctttgaaaaacacga

SEQ ID NO: 12 - DNA, 543 bp, Artificial Sequence
atggagcgggtgcagcccctggaggagaacgtgggcaacgccgccagacccaggttcgagagaaacaagctgctgctggtggccagcgtgatccagggactgggcctgctgctgtgcttcacctatatttgcctgcactttagtgccctgcaggtgagtcatagatacccccgcattcagtccatcaaagtgcagttcaccgagtataagaaggagaagggattcattctgacctcccagaaggaggacgagatcatgaaggtgcagaacaatagcgtgatcatcaactgtgacggcttttacctgatttcactgaaaggatacttcagccaggaggtgaatatcagcctgcactaccagaaagacgaggagcccctgttccagctgaagaaggtgaggagcgtgaacagcctgatggtggccagcctgacctacaaggacaaagtgtacctgaacgtgaccaccgacaacaccagcctggatgattttcacgtgaacggaggcgagctgatcctgatccatcagaaccccggcgagttctaa

SEQ ID NO: 13 - DNA, 4159 bp, Artificial Sequence
atgatcaagctgaagttcggggtgttcttcaccgtgctgctgagcagcgcctacgcccacgggacccctcagaacatcaccgacctgtgcgccgagtaccacaacacccagatctacaccctgaacgacaagattttcagctacaccgaaagcctggcaggaaaaagagagatggccatcatcaccttcaaaaacggcgccatcttccaggtggaggtgcccggcagccagcacatcgatagccagaagaaggccatcgaaagaatgaaggacacactgagaatcgcctacctgaccgaggccaaggtggaaaagctgtgcgtgtggaataataagaccccccacgccatcgccgccatcagcatggccaaccagtacatcaaggcaaacagcaaattcatcggaatcaccgaagccaaatttgtggccgcctggaccctgaaggcagccgctggcggcggcggcggcggccgcgtgcagcccaccgagagcatcgtgcgcttccccaacatcaccaacctgtgccccttcggcgaggtgttcaacgccacccgcttcgccagcgtgtacgcctggaaccgcaagcgcatcagcaactgcgtggccgactacagcgtgctgtacaacagcgccagcttcagcaccttcaagtgctacggcgtgagccccaccaagctgaacgacctgtgcttcaccaacgtgtacgccgacagcttcgtgatccgcggcgacgaggtgcgccagatcgcccccggccagaccggcaagatcgccgactacaactacaagctgcccgacgacttcaccggctgcgtgatcgcctggaacagcaacaacctggacagcaaggtgggcggcaactacaactacctgtaccgcctgttccgcaagagcaacctgaagcccttcgagcgcgacatcagcaccgagatctaccaggccggcagcaccccctgcaacggcgtggagggcttcaactgctacttccccctgcagagctacggcttccagcccaccaacggcgtgggctaccagccctaccgcgtggtggtgctgagcttcgagctgctgcacgcccccgccaccgtgtgcggccccaagaagagcaccaacctggtgaagaacaagtgcgtgaacttcggcggcggcggcagcggcggcggcggcagcgtgctgaacgacatcctgagccgcctggacaaggtggaggccgaggtgcagatcgaccgcctgatcaccggccgcctgcagagcctgcagacctacgtgacccagcagctgatccgcgccgccgagatccgcgccagcgccaacctggccgccaccaagatgagcgagtgcgtgctgggccagagcaagcgcgtggacttctgcggcaagggctaccacctgatgagcttcccccagagcgccccccacggcgtggtgttcctgcacgtgacctacgtgcccgcccaggagaagaacttcaccaccgcccccgccatctgccacgacggcaaggcccacttcccccgcgagggcgtgttcgtgagcaacggcacccactggttcgtgacccagcgcaacttctacgagccccagatcatcaccaccgacaacaccttcgtgagcggcaactgcgacgtggtgatcggcatcgtgaacaacaccgtgtacgaccccctgcagcccgagctggacagcttcaaggaggagctggacaagtacttcaagaaccacaccagccccgacgtggacctgggcgacatcagcggcatcaacgccagcgtggtgaacatccagaaggagatcgaccgcctgaacgaggtggccaagaacctgaacgagagcctgatcgacctgcaggagctgggcaagtacgagcagtacatcaagtggccctggtacatctggctgggcttcatcgccggcctgatcgccatcgtgatggtgaccatcatgctgtgctgcatgaccagctgctgcagctgcctgaagggctgctgcagctgcggcagctgctgcaagttcgacgaggacgacagcgagcccgtgctgaagggcgtgaagctgcactacaccggctacatccccgaggccccccgcgacggccaggcctacgtgcgcaaggacggcgagtgggtgctgctgagcaccttcctgtgccccccctgcccccgcgccaagcgcgcccccgtgaagcagaccctgaacttcgacctgctgaagctggccggcgacgtggagagcaaccccggccccatgcgctacatgatcctgggcctgctggccctggccgccgtgtgcagcgccgccctgaacacccccaaggaccacatcggcacccgcaaccccgccaacaacgccgccatcgtgctgcagctgccccagggcaccaccctgcccaagggcttctacgccgagggcagccgcggcggcagccaggccagcagccgcagcagcagccgcagccgcaacagcagccgcaacagcacccccggcagcagccgcggcaccagccccgcccgcatggccggcaacggcggcgacgccgccctggccctgctgctgctggaccgcctgaaccagctggagagcaagatgagcggcaagggccagcagcagcagggccagaccgtgaccaagaagagcgccgccgaggccagcaagaagccccgccagaagcgcaccgccaccaaggcctacaacgtgacccaggccttcggccgccgcggccccgagcagacccagggcaacttcggcgaccaggagctgatccgccagggcaccgactacaagcactggccccagatcgcccagttcgcccccagcgccagcgccttcttcggcatgagccgcatcggcatggaggtgacccccagcggcacctggctgacctacaccggcgccatcaagctggacgacaaggaccccaacttcaaggaccaggtgatcctgctgaacaagcacatcgacgcctacaagaccttcccccccaccgagcccaagtgagaattcggcccctctccctcccccccccctaacgttactggccgaagccgcttggaataaggccggtgtgcgtttgtctatatgttattttccaccatattgccgtcttttggcaatgtgagggcccggaaacctggccctgtcttcttgacgagcattcctaggggtctttcccctctcgccaaaggaatgcaaggtctgttgaatgtcgtgaaggaagcagttcctctggaagcttcttgaagacaaacaacgtctgtagcgaccctttgcaggcagcggaaccccccacctggcgacaggtgcctctgcggccaaaagccacgtgtataagatacacctgcaaaggcggcacaaccccagtgccacgttgtgagttggatagttgtggaaagagtcaaatggctctcctcaagcgtattcaacaaggggctgaaggatgcccagaaggtaccccattgtatgggatctgatctggggcctcggtgcacatgctttacatgtgtttagtcgaggttaaaaaaacgtctaggccccccgaaccacggggacgtggttttcctttgaaaaacacgatgataagcttgccacaacccgcgcgcttaattaacccggggccaccatggagcgggtgcagcccctggaggagaacgtgggcaacgccgccagacccaggttcgagagaaacaagctgctgctggtggccagcgtgatccagggactgggcctgctgctgtgcttcacctatatttgcctgcactttagtgccctgcaggtgagtcatagatacccccgcattcagtccatcaaagtgcagttcaccgagtataagaaggagaagggattcattctgacctcccagaaggaggacgagatcatgaaggtgcagaacaatagcgtgatcatcaactgtgacggcttttacctgatttcactgaaaggatacttcagccaggaggtgaatatcagcctgcactaccagaaagacgaggagcccctgttccagctgaagaaggtgaggagcgtgaacagcctgatggtggccagcctgacctacaaggacaaagtgtacctgaacgtgaccaccgacaacaccagcctggatgattttcacgtgaacggaggcgagctgatcctgatccatcagaaccccggcgagttctaa

SEQ ID NO: 14 - DNA, 31 bp, Artificial Sequence
cccaggagacccggttctagagacggacatt

SEQ ID NO: 15 - DNA, 31 bp, Artificial Sequence
aagcggcttcggccagtaacgttaggggggg